European Patent Specification EP 4 019 647 B1, published December 13, 2023. Title: MODIFIED MULTIPLEX AND MULTISTEP AMPLIFICATION REACTIONS AND REAGENTS THEREFOR. Applicant: Multiplicom N.V. Del Favero, Jurgen PL Heyrman, Lien Tegenbos, Bart Goossens, Dirk De Schrijver, Joachim. The sequence listing filed with the application follows.

SEQUENCE LISTING (24 sequences)

SEQ ID NO: 1 - DNA, 20 bp, Artificial Sequence
  Synthetic oligonucleotide
aagactcggcagcatctcca

SEQ ID NO: 2 - DNA, 20 bp, Artificial Sequence
  Synthetic oligonucleotide
gcgatcgtcactgttctcca

SEQ ID NO: 3 - DNA, 29 bp, Artificial Sequence
  Synthetic oligonucleotide
aatgatacggcgaccaccgagatctacac

SEQ ID NO: 4 - DNA, 24 bp, Artificial Sequence
  Synthetic oligonucleotide
caagcagaagacggcatacgagat

SEQ ID NO: 5 - DNA, 68 bp, Artificial Sequence
  Synthetic oligonucleotide
  misc_feature (1)..(19): reverse complement of Tag1
  misc_feature (21)..(39): MID sequence
  misc_feature (40)..(68): reverse complement of p5
ggagatgctgccgagtctttcctctgtcgacgtattgacgtgtagatctcggtggtcgccgtatcatt

SEQ ID NO: 6 - DNA, 68 bp, Artificial Sequence
  Synthetic oligonucleotide
  misc_feature (1)..(19): reverse complement of Tag1
  misc_feature (20)..(39): MID sequence
  misc_feature (40)..(68): reverse complement of p5
ggagatgctgccgagtctttcctctgtcgacactcaagtgtgtagatctcggtggtcgccgtatcatt

SEQ ID NO: 7 - DNA, 68 bp, Artificial Sequence
  Synthetic oligonucleotide
  misc_feature (1)..(19): reverse complement of Tag1
  misc_feature (20)..(39): MID sequence
  misc_feature (40)..(68): reverse complement of p5
ggagatgctgccgagtctttcctctgtcgacctcatgatgtgtagatctcggtggtcgccgtatcatt

SEQ ID NO: 8 - DNA, 68 bp, Artificial Sequence
  Synthetic oligonucleotide
  misc_feature (1)..(19): reverse complement of Tag1
  misc_feature (20)..(39): MID sequence
  misc_feature (40)..(68): reverse complement of p5
ggagatgctgccgagtctttcctctgtcgactcatatcggtgtagatctcggtggtcgccgtatcatt

SEQ ID NO: 9 - DNA, 68 bp, Artificial Sequence
  Synthetic oligonucleotide
  misc_feature (1)..(19): reverse complement of Tag1
  misc_feature (20)..(39): MID sequence
  misc_feature (40)..(68): reverse complement of p5
ggagatgctgccgagtctttcctctgtcgacctgccagagtgtagatctcggtggtcgccgtatcatt

SEQ ID NO: 10 - DNA, 68 bp, Artificial Sequence
  Synthetic oligonucleotide
  misc_feature (1)..(19): reverse complement of Tag1
  misc_feature (20)..(39): MID sequence
  misc_feature (40)..(68): reverse complement of p5
ggagatgctgccgagtctttcctctgtcgacgatggatagtgtagatctcggtggtcgccgtatcatt

SEQ ID NO: 11 - DNA, 68 bp, Artificial Sequence
  Synthetic oligonucleotide
  misc_feature (1)..(19): reverse complement of Tag1
  misc_feature (20)..(39): MID sequence
  misc_feature (40)..(68): reverse complement of p5
ggagatgctgccgagtctttcctctgtcgacctggacgggtgtagatctcggtggtcgccgtatcatt

SEQ ID NO: 12 - DNA, 68 bp, Artificial Sequence
  Synthetic oligonucleotide
  misc_feature (1)..(19): reverse complement of Tag1
  misc_feature (20)..(39): MID sequence
  misc_feature (40)..(68): reverse complement of p5
ggagatgctgccgagtctttcctctgtcgactcacggacgtgtagatctcggtggtcgccgtatcatt

SEQ ID NO: 13 - DNA, 68 bp, Artificial Sequence
  Synthetic oligonucleotide
  misc_feature (1)..(19): reverse complement of Tag1
  misc_feature (20)..(39): MID sequence
  misc_feature (40)..(68): reverse complement of p5
ggagatgctgccgagtctttcctctgtcgactatactaggtgtagatctcggtggtcgccgtatcatt

SEQ ID NO: 14 - DNA, 68 bp, Artificial Sequence
  Synthetic oligonucleotide
  misc_feature (1)..(19): reverse complement of Tag1
  misc_feature (20)..(39): MID sequence
  misc_feature (40)..(68): reverse complement of p5
ggagatgctgccgagtctttcctctgtcgacgcttgactgtgtagatctcggtggtcgccgtatcatt

SEQ ID NO: 15 - DNA, 67 bp, Artificial Sequence
  Synthetic oligonucleotide
  misc_feature (1)..(20): reverse complement of Tag2
  misc_feature (21)..(43): MID sequence
  misc_feature (44)..(67): reverse complement of p7
ggagaacagtgacgatcgcttgggacctaggtaatggaggaacatctcgtatgccgtcttctgcttg

SEQ ID NO: 16 - DNA, 67 bp, Artificial Sequence
  Synthetic oligonucleotide
  misc_feature (1)..(19): reverse complement of Tag2
  misc_feature (20)..(43): MID sequence
  misc_feature (44)..(67): reverse complement of p7
ggagaacagtgacgatcgcttgggacctaggtgatagtgaggaatctcgtatgccgtcttctgcttg

SEQ ID NO: 17 - DNA, 67 bp, Artificial Sequence
  Synthetic oligonucleotide
  misc_feature (1)..(19): reverse complement of Tag2
  misc_feature (20)..(43): MID sequence
  misc_feature (44)..(67): reverse complement of p7
ggagaacagtgacgatcgcttgggacctaggatcaaagggcaaatctcgtatgccgtcttctgcttg

SEQ ID NO: 18 - DNA, 67 bp, Artificial Sequence
  Synthetic oligonucleotide
  misc_feature (1)..(19): reverse complement of Tag2
  misc_feature (20)..(43): MID sequence
  misc_feature (44)..(67): reverse complement of p7
ggagaacagtgacgatcgcttgggacctaggcaccgggaatcaatctcgtatgccgtcttctgcttg

SEQ ID NO: 19 - DNA, 67 bp, Artificial Sequence
  Synthetic oligonucleotide
  misc_feature (1)..(19): reverse complement of Tag2
  misc_feature (20)..(43): MID sequence
  misc_feature (44)..(67): reverse complement of p7
ggagaacagtgacgatcgcttgggacctaggccgtagtttaggatctcgtatgccgtcttctgcttg

SEQ ID NO: 20 - DNA, 67 bp, Artificial Sequence
  Synthetic oligonucleotide
  misc_feature (1)..(19): reverse complement of Tag2
  misc_feature (20)..(43): MID sequence
  misc_feature (44)..(67): reverse complement of p7
ggagaacagtgacgatcgcttgggacctaggtgtcgaaagagaatctcgtatgccgtcttctgcttg

SEQ ID NO: 21 - DNA, 67 bp, Artificial Sequence
  Synthetic oligonucleotide
  misc_feature (1)..(19): reverse complement of Tag2
  misc_feature (20)..(43): MID sequence
  misc_feature (44)..(67): reverse complement of p7
ggagaacagtgacgatcgcttgggacctaggactgccattaacatctcgtatgccgtcttctgcttg

SEQ ID NO: 22 - DNA, 67 bp, Artificial Sequence
  Synthetic oligonucleotide
  misc_feature (1)..(19): reverse complement of Tag2
  misc_feature (20)..(43): MID sequence
  misc_feature (44)..(67): reverse complement of p7
ggagaacagtgacgatcgcttgggacctaggttggccacttccatctcgtatgccgtcttctgcttg

SEQ ID NO: 23 - DNA, 67 bp, Artificial Sequence
  Synthetic oligonucleotide
  misc_feature (1)..(19): reverse complement of Tag2
  misc_feature (20)..(43): MID sequence
  misc_feature (44)..(67): reverse complement of p7
ggagaacagtgacgatcgcttgggacctaggattcctgtgagtatctcgtatgccgtcttctgcttg

SEQ ID NO: 24 - DNA, 67 bp, Artificial Sequence
  Synthetic oligonucleotide
  misc_feature (1)..(19): reverse complement of Tag2
  misc_feature (20)..(43): MID sequence
  misc_feature (44)..(67): reverse complement of p7
ggagaacagtgacgatcgcttgggacctaggccatggacacagatctcgtatgccgtcttctgcttg